European Patent Specification EP 4 003 533 B1, published March 13, 2024. Title: METHODS OF TREATING MULTIFOCAL CANCER. Applicant: NYMOX CORPORATION AVERBACK, Paul. The sequence listing filed with the application follows.

SEQUENCE LISTING (1 sequence)

SEQ ID NO: 1 - protein, 17 aa, Artificial Sequence
  Synthetic peptide
IDQQVLSRIKLEIKRCL